European Patent Application EP 4 681 724 A1, published January 21, 2026. Title: 抑制过激炎性反应的蛋白及其应用. Applicant: 中国科学院上海巴斯德研究所. The sequence listing filed with the application follows.

SEQUENCE LISTING (4 sequences)

SEQ ID NO: 1 - protein, 394 aa, Mus musculus
MCRAISLRRLLLLLLQLSQLLAVTQGKTLVLGKEGESAELPCESSQKKITVFTWKFSDQRKILGQHGKGVLIRGGSPSQFDRFDSKKGAWEKGSFPLIINKLKMEDSQTYICELENRKEEVELWVFKVTFSPGTSLLQGQSLTLTLDSNSKVSNPLTECKHKKGKVVSGSKVLSMSNLRVQDSDFWNCTVTLDQKKNWFGMTLSVLGFQSTAITAYKSEGESAEFSFPLNFAEENGWGELMWKAEKDSFFQPWISFSIKNKEVSVQKSTKDLKLQLKETLPLTLKIPQVSLQFAGSGNLTLTLDKGTLHQEVNLVVMKVAQLNNTLTCEVMGPTSPKMRLTLKQENQEARVSEEQKVVQVVAPETGLWQCLLSEGDKVKMDSRIQVLSRGVNQT

SEQ ID NO: 2 - DNA, 1182 bp, Mus musculus
  source 1..1182: mol_type = other DNA
atgtgccgagccatctctcttaggcgcttgctgctgctgctgctgcagctgtcacaactcctagctgtcactcaagggaagacgctggtgctggggaaggaaggggaatcagcagaactgccctgcgagagttcccagaagaagatcacagtcttcacctggaagttctctgaccagaggaagattctggggcagcatggcaaaggtgtattaattagaggaggttcgccttcgcagtttgatcgttttgattccaaaaaaggggcatgggagaaaggatcgtttcctctcatcatcaataaacttaagatggaagactctcagacttatatctgtgagctggagaacaggaaagaggaggtggagttgtgggtgttcaaagtgaccttcagtccgggtaccagcctgttgcaagggcagagcctgaccctgaccttggatagcaactctaaggtctctaaccccttgacagagtgcaaacacaaaaagggtaaagttgtcagtggttccaaagttctctccatgtccaacctaagggttcaggacagcgacttctggaactgcaccgtgaccctggaccagaaaaagaactggttcggcatgacactctcagtgctgggttttcagagcacagctatcacggcctataagagtgagggagagtcagcggagttctccttcccactcaactttgcagaggaaaacgggtggggagagctgatgtggaaggcagagaaggattctttcttccagccctggatctccttctccataaagaacaaagaggtgtccgtacaaaagtccaccaaagacctcaagctccagctgaaggaaacgctcccactcaccctcaagataccccaggtctcgcttcagtttgctggttctggcaacctgactctgactctggacaaagggacactgcatcaggaagtgaacctggtggtgatgaaagtggctcagctcaacaatactttgacctgtgaggtgatgggacctacctctcccaagatgagactgaccctgaagcaggagaaccaggaggccagggtctctgaggagcagaaagtagttcaagtggtggcccctgagacagggctgtggcagtgtctactgagtgaaggtgataaggtcaagatggactccaggatccaggttttatccagaggggtgaaccagaca

SEQ ID NO: 3 - protein, 412 aa, Homo sapiens
MNRGVPFRHLLLVLQLALLPAATQGKKVVLGKKGDTVELTCTASQKKSIQFHWKNSNQIKILGNQGSFLTKGPSKLNDRADSRRSLWDQGNFPLIIKNLKIEDSDTYICEVEDQKEEVQLLVFGLTANSDTHLLQGQSLTLTLESPPGSSPSVQCRSPRGKNIQGGKTLSVSQLELQDSGTWTCTVLQNQKKVEFKIDIVVLAFQKASSIVYKKEGEQVEFSFPLAFTVEKLTGSGELWWQAERASSSKSWITFDLKNKEVSVKRVTQDPKLQMGKKLPLHLTLPQALPQYAGSGNLTLALEAKTGKLHQEVNLVVMRATQLQKNLTCEVWGPTSPKLMLSLKLENKEAKVSKREKAVWVLNPEAGMWQCLLSDSGQVLLESNIKVLPTWSTPVQPMALIVLGGVAGLLLFI

SEQ ID NO: 4 - DNA, 1236 bp, Homo sapiens
  source 1..1236: mol_type = other DNA
ctctcttcatttaagcacgactctgcagaaggaacaaagcaccctccccactgggctcctggttgcagagctccaagtcctcacacagatacgcctgtttgagaagcagcgggcaagaaagacgcaagcccagaggccctgccatttctgtgggctcaggtccctactggctcaggcccctgcctccctcggcaaggccacaatgaaccggggagtcccttttaggcacttgcttctggtgctgcaactggcgctcctcccagcagccactcagggaaagaaagtggtgctgggcaaaaaaggggatacagtggaactgacctgtacagcttcccagaagaagagcatacaattccactggaaaaactccaaccagataaagattctgggaaatcagggctccttcttaactaaaggtccatccaagctgaatgatcgcgctgactcaagaagaagcctttgggaccaaggaaactttcccctgatcatcaagaatcttaagatagaagactcagatacttacatctgtgaagtggaggaccagaaggaggaggtgcaattgctagtgttcggattgactgccaactctgacacccacctgcttcaggggcagagcctgaccctgaccttggagagcccccctggtagtagcccctcagtgcaatgtaggagtccaaggggtaaaaacatacagggggggaagaccctctccgtgtctcagctggagctccaggatagtggcacctggacatgcactgtcttgcagaaccagaagaaggtggagttcaaaatagacatcgtggtgctagctttccagaaggcctccagcatagtctataagaaagagggggaacaggtggagttctccttcccactcgcctttacagttgaaaagctgacgggcagtggcgagctgtggtggcaggcggagagggcttcctcctccaagtcttggatcacctttgacctgaagaacaaggaagtgtctgtaaaacgggttacccaggaccctaagctccagatgggcaagaagctcccgctccacctcaccctgccccaggccttgcctcagtatgctggctctggaaacctcaccctggcccttgaagcgaaaacaggaaagttgcatcaggaagtgaacctggtggtgatgagagccactcagctccagaaaaatttgacctgtgaggtgtggggacccacctcccctaagctgatgctgagtttgaaactgga